European Patent Specification EP 3 801 010 B1, published January 1, 2025. Title: Transgenic Animal For Producing Diversified Antibodies That Have The Same Light Chain. Applicant: Crystal Bioscience Inc. Leighton, Philip A Harriman, William  Don Etches, Robert. The sequence listing filed with the application follows.

SEQUENCE LISTING (2 sequences)

SEQ ID NO: 1 - protein, 108 aa, Artificial sequence
  synthetic sequence
EIVMTQSPATLSVSPGERATLSCRASQSVSSNLAWYQQKPGQAPRLLIYGASTRATGIPARFSGSGSGTEFTLTISSLQSEDFAVYYCQQYNNWPPWTFGQGTKVEIK

SEQ ID NO: 2 - protein, 128 aa, Artificial sequence
  synthetic sequence
MAAVTLDESGGGLQTPGRALSLVCKASGFTFSSYNMGWVRQAPGKGLEFVAGIDNTGRYTGYGSAVKGRATISRDNGQSTVRLQLLRAEDTNNGTYYCAKAAGDLGYGDLYAGQIDAWGHGTEVIVSS